European Patent Specification EP 3 806 884 B1, published August 2, 2023. Title: GENERAL AMYLOID INTERACTION MOTIF (GAIM). Applicant: PROCLARA BIOSCIENCES, INC. The sequence listing filed with the application follows.

SEQUENCE LISTING (54 sequences)

SEQ ID NO: 1 - protein, 32 aa, Artificial Sequence
  source: /note="Description of Artificial Sequence: Synthetic polypeptide"
AETVESCLAKPHTENSFTNVWKDDKTLDRYAN

SEQ ID NO: 2 - protein, 30 aa, Artificial Sequence
  source: /note="Description of Artificial Sequence: Synthetic polypeptide"
ATTDAECLSKPAFDGTLSNVWKEGDSRYAN

SEQ ID NO: 3 - protein, 6 aa, Artificial Sequence
  source: /note="Description of Artificial Sequence: Synthetic peptide"
DDKTLD

SEQ ID NO: 4 - protein, 4 aa, Artificial Sequence
  source: /note="Description of Artificial Sequence: Synthetic peptide"
EGDS

SEQ ID NO: 5 - protein, 4 aa, Artificial Sequence
  source: /note="Description of Artificial Sequence: Synthetic peptide"
FQNN

SEQ ID NO: 6 - protein, 4 aa, Artificial Sequence
  source: /note="Description of Artificial Sequence: Synthetic peptide"
RQGA

SEQ ID NO: 7 - protein, 7 aa, Artificial Sequence
  source: /note="Description of Artificial Sequence: Synthetic peptide"
QGTDPVK

SEQ ID NO: 8 - protein, 4 aa, Artificial Sequence
  source: /note="Description of Artificial Sequence: Synthetic peptide"
FQGN

SEQ ID NO: 9 - protein, 4 aa, Artificial Sequence
  source: /note="Description of Artificial Sequence: Synthetic peptide"
VNGV

SEQ ID NO: 10 - protein, 4 aa, Artificial Sequence
  source: /note="Description of Artificial Sequence: Synthetic peptide"
QGGK

SEQ ID NO: 11 - protein, 487 aa, Artificial Sequence
  source: /note="Description of Artificial Sequence: Synthetic polypeptide"
MAETVESCLAKPHTENSFTNVWKDDKTLDRYANYEGCLWNAGGVVVCTGDETQCYGTWVPIGLAIPENEGGGSEGGGSEGGGSEGGGTKPPEYGDTPIPGYTYINPLDGTYPPGTEQNPANPNPSLEESQPLNTFMFQNNRFRNRQGALTVYTGTFTQGTDPVKTYYQYTPVSSRAMYDAYWNGKFRDCAFHSGFNEDPFVCEYQGQSSDLPQPPANAGGESGGGSGGGSEGGGSEGGGSEGGGSEGGGSGGGSGSGARSDKTHTCPPCPAPELLGGPSVFLFPPKPKDTLMISRTPEVTCVVVDVSHEDPEVKFNWYVDGVEVHNAKTKPREEQYNSTYRVVSVLTVLHQDWLNGKEYKCKVSNKALPAPIEKTISKAKGQPREPQVYTLPPSREEMTKNQVSLTCLVKGFYPSDIAVEWESNGQPENNYKTTPPVLDSDGSFFLYSKLTVDKSRWQQGNVFSCSVMHEALHNHYTQKSLSLSPGK

SEQ ID NO: 12 - protein, 257 aa, Artificial Sequence
  source: /note="Description of Artificial Sequence: Synthetic polypeptide"
MAETVESCLAKPHTENSFTNVWKDDKTLDRYANYEGCLWNAGGVVVCTGDETQCYGTWVPIGLAIPENEGGGSEGGGSEGGGSEGGGTKPPEYGDTPIPGYTYINPLDGTYPPGTEQNPANPNPSLEESQPLNTFMFQNNRFRNRQGALTVYTGTFTQGTDPVKTYYQYTPVSSRAMYDAYWNGKFRDCAFHSGFNEDPFVCEYQGQSSDLPQPPANAGGESGGGSGGGSEGGGSEGGGSEGGGSEGGGSGGGSGSG

SEQ ID NO: 13 - protein, 487 aa, Artificial Sequence
  source: /note="Description of Artificial Sequence: Synthetic polypeptide"
MAETVESCLAKPHTENSFTNVWKDDKTLDRYANYEGCLWNAGGVVVCTGDETQCYGHWVPIGLAIPENEGGGSEGGGSEGGGSEGGGTKPPEYGDTPIPGYTYINPLDGTYPPGTEQNPANPNPSLEESQPLNTFMFQNNRFRNRQGALTVYTGTFTQGTDPVKTYYQYTPVSSRAMYDAYWNGKFRDCAFHSGFNEDPFVCEYQGQSSDLPQPPANAGGESGGGSGGGSEGGGSEGGGSEGGGSEGGGSGGGSGSGARSDKTHTCPPCPAPELLGGPSVFLFPPKPKDTLMISRTPEVTCVVVDVSHEDPEVKFNWYVDGVEVHNAKTKPREEQYNSTYRVVSVLTVLHQDWLNGKEYKCKVSNKALPAPIEKTISKAKGQPREPQVYTLPPSREEMTKNQVSLTCLVKGFYPSDIAVEWESNGQPENNYKTTPPVLDSDGSFFLYSKLTVDKSRWQQGNVFSCSVMHEALHNHYTQKSLSLSPGK

SEQ ID NO: 14 - protein, 257 aa, Artificial Sequence
  source: /note="Description of Artificial Sequence: Synthetic polypeptide"
MAETVESCLAKPHTENSFTNVWKDDKTLDRYANYEGCLWNAGGVVVCTGDETQCYGHWVPIGLAIPENEGGGSEGGGSEGGGSEGGGTKPPEYGDTPIPGYTYINPLDGTYPPGTEQNPANPNPSLEESQPLNTFMFQNNRFRNRQGALTVYTGTFTQGTDPVKTYYQYTPVSSRAMYDAYWNGKFRDCAFHSGFNEDPFVCEYQGQSSDLPQPPANAGGESGGGSGGGSEGGGSEGGGSEGGGSEGGGSGGGSGSG

SEQ ID NO: 15 - protein, 485 aa, Artificial Sequence
  source: /note="Description of Artificial Sequence: Synthetic polypeptide"
MAETVESCLAKPHTENSFTNVWKEGDSRYANYEGCLWNAGGVVVCTGDETQCYGHWVPIGLAIPENEGGGSEGGGSEGGGSEGGGTKPPEYGDTPIPGYTYINPLDGTYPPGTEQNPANPNPSLEESQPLNTFMFQNNRFRNRQGALTVYTGTFTQGTDPVKTYYQYTPVSSRAMYDAYWNGKFRDCAFHSGFNEDPFVCEYQGQSSDLPQPPANAGGESGGGSGGGSEGGGSEGGGSEGGGSEGGGSGGGSGSGARSDKTHTCPPCPAPELLGGPSVFLFPPKPKDTLMISRTPEVTCVVVDVSHEDPEVKFNWYVDGVEVHNAKTKPREEQYNSTYRVVSVLTVLHQDWLNGKEYKCKVSNKALPAPIEKTISKAKGQPREPQVYTLPPSREEMTKNQVSLTCLVKGFYPSDIAVEWESNGQPENNYKTTPPVLDSDGSFFLYSKLTVDKSRWQQGNVFSCSVMHEALHNHYTQKSLSLSPGK

SEQ ID NO: 16 - protein, 255 aa, Artificial Sequence
  source: /note="Description of Artificial Sequence: Synthetic polypeptide"
MAETVESCLAKPHTENSFTNVWKEGDSRYANYEGCLWNAGGVVVCTGDETQCYGHWVPIGLAIPENEGGGSEGGGSEGGGSEGGGTKPPEYGDTPIPGYTYINPLDGTYPPGTEQNPANPNPSLEESQPLNTFMFQNNRFRNRQGALTVYTGTFTQGTDPVKTYYQYTPVSSRAMYDAYWNGKFRDCAFHSGFNEDPFVCEYQGQSSDLPQPPANAGGESGGGSGGGSEGGGSEGGGSEGGGSEGGGSGGGSGSG

SEQ ID NO: 17 - protein, 487 aa, Artificial Sequence
  source: /note="Description of Artificial Sequence: Synthetic polypeptide"
MAETVESSLAKPHIEGSFTNVWKDDKTLDWYANYEGILWKATGVVVITGDETQVYAIWVPVGLAIPENEGGGSEGGGSEGGGSEGGGTKPPEYGDTPIPGYIYINPLDGTYPPGTEQNPANPNPSLEESHPLNTFMFQGNRFRNRQGALTVYTGTFTQGTDPVKTYYQYTPVSSRAMYDAYWNGKFRDVAFHSGFNEDPLVAEYQGQLSYLPQPPANAGGESGGGSGGGSEGGGSEGGGSEGGGSEGGGSGGGSGSGARSDKTHTCPPCPAPELLGGPSVFLFPPKPKDTLMISRTPEVTCVVVDVSHEDPEVKFNWYVDGVEVHNAKTKPREEQYNSTYRVVSVLTVLHQDWLNGKEYKCKVSNKALPAPIEKTISKAKGQPREPQVYTLPPSREEMTKNQVSLTCLVKGFYPSDIAVEWESNGQPENNYKTTPPVLDSDGSFFLYSKLTVDKSRWQQGNVFSCSVMHEALHNHYTQKSLSLSPGK

SEQ ID NO: 18 - protein, 257 aa, Artificial Sequence
  source: /note="Description of Artificial Sequence: Synthetic polypeptide"
MAETVESSLAKPHIEGSFTNVWKDDKTLDWYANYEGILWKATGVVVITGDETQVYAIWVPVGLAIPENEGGGSEGGGSEGGGSEGGGTKPPEYGDTPIPGYIYINPLDGTYPPGTEQNPANPNPSLEESHPLNTFMFQGNRFRNRQGALTVYTGTFTQGTDPVKTYYQYTPVSSRAMYDAYWNGKFRDVAFHSGFNEDPLVAEYQGQLSYLPQPPANAGGESGGGSGGGSEGGGSEGGGSEGGGSEGGGSGGGSGSG

SEQ ID NO: 19 - protein, 255 aa, Artificial Sequence
  source: /note="Description of Artificial Sequence: Synthetic polypeptide"
MAETVESCLAKPHTENSFTNVWKEGDSRYANYEGCLWNAGGVVVCTGDETQCYGHWVPIGLAIPENEGGGSEGGGSEGGGSEGGGTKPPEYGDTPIPGYTYINPLDGTYPPGTEQNPANPNPSLEESQPLNTFMFQGNRFRNRQGALTVYTGTFTQGTDPVKTYYQYTPVSSRAMYDAYWNGKFRDCAFHSGFNEDPFVCEYQGQSSDLPQPPANAGGESGGGSGGGSEGGGSEGGGSEGGGSEGGGSGGGSGSG

SEQ ID NO: 20 - protein, 255 aa, Artificial Sequence
  source: /note="Description of Artificial Sequence: Synthetic polypeptide"
MAETVESCLAKPHTENSFTNVWKEGDSRYANYEGCLWNAGGVVVCTGDETQCYGHWVPIGLAIPENEGGGSEGGGSEGGGSEGGGTKPPEYGDTPIPGYTYINPLDGTYPPGTEQNPANPNPSLEESQPLNTFMFQNNRFRNVNGVLTVYTGTFTQGTDPVKTYYQYTPVSSRAMYDAYWNGKFRDCAFHSGFNEDPFVCEYQGQSSDLPQPPANAGGESGGGSGGGSEGGGSEGGGSEGGGSEGGGSGGGSGSG

SEQ ID NO: 21 - protein, 255 aa, Artificial Sequence
  source: /note="Description of Artificial Sequence: Synthetic polypeptide"
MAETVESCLAKPHTENSFTNVWKEGDSRYANYEGCLWNAGGVVVCTGDETQCYGHWVPIGLAIPENEGGGSEGGGSEGGGSEGGGTKPPEYGDTPIPGYTYINPLDGTYPPGTEQNPANPNPSLEESQPLNTFMFQGNRFRARQGALTVYTGTFTQGTDPVKTYYQYTPVSSRAMYDAYWNGKFRDCAFHSGFNEDPFVCEYQGQSSDLPQPPANAGGESGGGSGGGSEGGGSEGGGSEGGGSEGGGSGGGSGSG

SEQ ID NO: 22 - protein, 255 aa, Artificial Sequence
  source: /note="Description of Artificial Sequence: Synthetic polypeptide"
MAETVESCLAKPHTENSFTNVWKEGDSRYANYEGCLWNAGGVVVCTGDETQCYGHWVPIGLAIPENEGGGSEGGGSEGGGSEGGGTKPPEYGDTPIPGYTYINPLDGTYPPGTEQNPANPNPSLEESQPLNTFMFQNNRFRAVNGVLTVYTGTFTQGTDPVKTYYQYTPVSSRAMYDAYWNGKFRDCAFHSGFNEDPFVCEYQGQSSDLPQPPANAGGESGGGSGGGSEGGGSEGGGSEGGGSEGGGSGGGSGSG

SEQ ID NO: 23 - protein, 255 aa, Artificial Sequence
  source: /note="Description of Artificial Sequence: Synthetic polypeptide"
MAETVESCLAKPHTENSFTNVWKEGDSRYANYEGCLWNAGGVVVCTGDEHQCYGTWVPIGLAIPENEGGGSEGGGSEGGGSEGGGTKPPEYGDTPIPGYTYINPLDGTYPPGTEQNPANPNPSLEESQPLNTFMFQGNRFRARQGALTVYTGTFTQGTDPVKTYYQYTPVSSRAMYDAYWNGKFRDCAFHSGFNEDPFVCEYQGQSSDLPQPPANAGGESGGGSGGGSEGGGSEGGGSEGGGSEGGGSGGGSGSG

SEQ ID NO: 24 - protein, 255 aa, Artificial Sequence
  source: /note="Description of Artificial Sequence: Synthetic polypeptide"
MAETVESCLAKPHTENSFTNVWKEGDSRYANYEGCLWNAGGVVVCTGDEHQCYGTWVPIGLAIPENEGGGSEGGGSEGGGSEGGGTKPPEYGDTPIPGYTYINPLDGTYPPGTEQNPANPNPSLEESQPLNTFMFQNNRFRAVNGVLTVYTGTFTQGTDPVKTYYQYTPVSSRAMYDAYWNGKFRDCAFHSGFNEDPFVCEYQGQSSDLPQPPANAGGESGGGSGGGSEGGGSEGGGSEGGGSEGGGSGGGSGSG

SEQ ID NO: 25 - protein, 255 aa, Artificial Sequence
  source: /note="Description of Artificial Sequence: Synthetic polypeptide"
MAETVESCLAKPHTENSFTNVWKEGDSRYANYEGCLWNAGGVVVCTGDEHQCYGTWVPIGLAIPENEGGGSEGGGSEGGGSEGGGTKPPEYGDTPIPGYTYINPLDGTYPPGTEQNPANPNPSLEESQPLNTFMFQGNRFRNRQGALTVYTGTFTQGTDPVKTYYQYTPVSSRAMYDAYWNGKFRDCAFHSGFNEDPFVCEYQGQSSDLPQPPANAGGESGGGSGGGSEGGGSEGGGSEGGGSEGGGSGGGSGSG

SEQ ID NO: 26 - protein, 255 aa, Artificial Sequence
  source: /note="Description of Artificial Sequence: Synthetic polypeptide"
MAETVESCLAKPHTENSFTNVWKEGDSRYANYEGCLWAAGGVVVCTGDEHQCYGTWVPIGLAIPENEGGGSEGGGSEGGGSEGGGTKPPEYGDTPIPGYTYINPLDGTYPPGTEQNPANPNPSLEESQPLNTFMFQGNRFRNRQGALTVYTGTFTQGTDPVKTYYQYTPVSSRAMYDAYWNGKFRDCAFHSGFNEDPFVCEYQGQSSDLPQPPANAGGESGGGSGGGSEGGGSEGGGSEGGGSEGGGSGGGSGSG

SEQ ID NO: 27 - protein, 5 aa, Artificial Sequence
  source: /note="Description of Artificial Sequence: Synthetic peptide"
GGGGS

SEQ ID NO: 28 - protein, 4 aa, Artificial Sequence
  source: /note="Description of Artificial Sequence: Synthetic peptide"
GGGS

SEQ ID NO: 29 - protein, 485 aa, Artificial Sequence
  source: /note="Description of Artificial Sequence: Synthetic polypeptide"
MAETVESCLAKPHTENSFTNVWKEGDSRYANYEGCLWNAGGVVVCTGDETQCYGHWVPIGLAIPENEGGGSEGGGSEGGGSEGGGTKPPEYGDTPIPGYTYINPLDGTYPPGTEQNPANPNPSLEESQPLNTFMFQGNRFRNRQGALTVYTGTFTQGTDPVKTYYQYTPVSSRAMYDAYWNGKFRDCAFHSGFNEDPFVCEYQGQSSDLPQPPANAGGESGGGSGGGSEGGGSEGGGSEGGGSEGGGSGGGSGSGARSDKTHTCPPCPAPELLGGPSVFLFPPKPKDTLMISRTPEVTCVVVDVSHEDPEVKFNWYVDGVEVHNAKTKPREEQYNSTYRVVSVLTVLHQDWLNGKEYKCKVSNKALPAPIEKTISKAKGQPREPQVYTLPPSREEMTKNQVSLTCLVKGFYPSDIAVEWESNGQPENNYKTTPPVLDSDGSFFLYSKLTVDKSRWQQGNVFSCSVMHEALHNHYTQKSLSLSPGK

SEQ ID NO: 30 - protein, 485 aa, Artificial Sequence
  source: /note="Description of Artificial Sequence: Synthetic polypeptide"
MAETVESCLAKPHTENSFTNVWKEGDSRYANYEGCLWNAGGVVVCTGDETQCYGHWVPIGLAIPENEGGGSEGGGSEGGGSEGGGTKPPEYGDTPIPGYTYINPLDGTYPPGTEQNPANPNPSLEESQPLNTFMFQNNRFRNVNGVLTVYTGTFTQGTDPVKTYYQYTPVSSRAMYDAYWNGKFRDCAFHSGFNEDPFVCEYQGQSSDLPQPPANAGGESGGGSGGGSEGGGSEGGGSEGGGSEGGGSGGGSGSGARSDKTHTCPPCPAPELLGGPSVFLFPPKPKDTLMISRTPEVTCVVVDVSHEDPEVKFNWYVDGVEVHNAKTKPREEQYNSTYRVVSVLTVLHQDWLNGKEYKCKVSNKALPAPIEKTISKAKGQPREPQVYTLPPSREEMTKNQVSLTCLVKGFYPSDIAVEWESNGQPENNYKTTPPVLDSDGSFFLYSKLTVDKSRWQQGNVFSCSVMHEALHNHYTQKSLSLSPGK

SEQ ID NO: 31 - protein, 485 aa, Artificial Sequence
  source: /note="Description of Artificial Sequence: Synthetic polypeptide"
MAETVESCLAKPHTENSFTNVWKEGDSRYANYEGCLWNAGGVVVCTGDETQCYGHWVPIGLAIPENEGGGSEGGGSEGGGSEGGGTKPPEYGDTPIPGYTYINPLDGTYPPGTEQNPANPNPSLEESQPLNTFMFQGNRFRARQGALTVYTGTFTQGTDPVKTYYQYTPVSSRAMYDAYWNGKFRDCAFHSGFNEDPFVCEYQGQSSDLPQPPANAGGESGGGSGGGSEGGGSEGGGSEGGGSEGGGSGGGSGSGARSDKTHTCPPCPAPELLGGPSVFLFPPKPKDTLMISRTPEVTCVVVDVSHEDPEVKFNWYVDGVEVHNAKTKPREEQYNSTYRVVSVLTVLHQDWLNGKEYKCKVSNKALPAPIEKTISKAKGQPREPQVYTLPPSREEMTKNQVSLTCLVKGFYPSDIAVEWESNGQPENNYKTTPPVLDSDGSFFLYSKLTVDKSRWQQGNVFSCSVMHEALHNHYTQKSLSLSPGK

SEQ ID NO: 32 - protein, 485 aa, Artificial Sequence
  source: /note="Description of Artificial Sequence: Synthetic polypeptide"
MAETVESCLAKPHTENSFTNVWKEGDSRYANYEGCLWNAGGVVVCTGDETQCYGHWVPIGLAIPENEGGGSEGGGSEGGGSEGGGTKPPEYGDTPIPGYTYINPLDGTYPPGTEQNPANPNPSLEESQPLNTFMFQNNRFRAVNGVLTVYTGTFTQGTDPVKTYYQYTPVSSRAMYDAYWNGKFRDCAFHSGFNEDPFVCEYQGQSSDLPQPPANAGGESGGGSGGGSEGGGSEGGGSEGGGSEGGGSGGGSGSGARSDKTHTCPPCPAPELLGGPSVFLFPPKPKDTLMISRTPEVTCVVVDVSHEDPEVKFNWYVDGVEVHNAKTKPREEQYNSTYRVVSVLTVLHQDWLNGKEYKCKVSNKALPAPIEKTISKAKGQPREPQVYTLPPSREEMTKNQVSLTCLVKGFYPSDIAVEWESNGQPENNYKTTPPVLDSDGSFFLYSKLTVDKSRWQQGNVFSCSVMHEALHNHYTQKSLSLSPGK

SEQ ID NO: 33 - protein, 485 aa, Artificial Sequence
  source: /note="Description of Artificial Sequence: Synthetic polypeptide"
MAETVESCLAKPHTENSFTNVWKEGDSRYANYEGCLWNAGGVVVCTGDEHQCYGTWVPIGLAIPENEGGGSEGGGSEGGGSEGGGTKPPEYGDTPIPGYTYINPLDGTYPPGTEQNPANPNPSLEESQPLNTFMFQGNRFRARQGALTVYTGTFTQGTDPVKTYYQYTPVSSRAMYDAYWNGKFRDCAFHSGFNEDPFVCEYQGQSSDLPQPPANAGGESGGGSGGGSEGGGSEGGGSEGGGSEGGGSGGGSGSGARSDKTHTCPPCPAPELLGGPSVFLFPPKPKDTLMISRTPEVTCVVVDVSHEDPEVKFNWYVDGVEVHNAKTKPREEQYNSTYRVVSVLTVLHQDWLNGKEYKCKVSNKALPAPIEKTISKAKGQPREPQVYTLPPSREEMTKNQVSLTCLVKGFYPSDIAVEWESNGQPENNYKTTPPVLDSDGSFFLYSKLTVDKSRWQQGNVFSCSVMHEALHNHYTQKSLSLSPGK

SEQ ID NO: 34 - protein, 485 aa, Artificial Sequence
  source: /note="Description of Artificial Sequence: Synthetic polypeptide"
MAETVESCLAKPHTENSFTNVWKEGDSRYANYEGCLWNAGGVVVCTGDEHQCYGTWVPIGLAIPENEGGGSEGGGSEGGGSEGGGTKPPEYGDTPIPGYTYINPLDGTYPPGTEQNPANPNPSLEESQPLNTFMFQNNRFRAVNGVLTVYTGTFTQGTDPVKTYYQYTPVSSRAMYDAYWNGKFRDCAFHSGFNEDPFVCEYQGQSSDLPQPPANAGGESGGGSGGGSEGGGSEGGGSEGGGSEGGGSGGGSGSGARSDKTHTCPPCPAPELLGGPSVFLFPPKPKDTLMISRTPEVTCVVVDVSHEDPEVKFNWYVDGVEVHNAKTKPREEQYNSTYRVVSVLTVLHQDWLNGKEYKCKVSNKALPAPIEKTISKAKGQPREPQVYTLPPSREEMTKNQVSLTCLVKGFYPSDIAVEWESNGQPENNYKTTPPVLDSDGSFFLYSKLTVDKSRWQQGNVFSCSVMHEALHNHYTQKSLSLSPGK

SEQ ID NO: 35 - protein, 485 aa, Artificial Sequence
  source: /note="Description of Artificial Sequence: Synthetic polypeptide"
MAETVESCLAKPHTENSFTNVWKEGDSRYANYEGCLWNAGGVVVCTGDEHQCYGTWVPIGLAIPENEGGGSEGGGSEGGGSEGGGTKPPEYGDTPIPGYTYINPLDGTYPPGTEQNPANPNPSLEESQPLNTFMFQGNRFRNRQGALTVYTGTFTQGTDPVKTYYQYTPVSSRAMYDAYWNGKFRDCAFHSGFNEDPFVCEYQGQSSDLPQPPANAGGESGGGSGGGSEGGGSEGGGSEGGGSEGGGSGGGSGSGARSDKTHTCPPCPAPELLGGPSVFLFPPKPKDTLMISRTPEVTCVVVDVSHEDPEVKFNWYVDGVEVHNAKTKPREEQYNSTYRVVSVLTVLHQDWLNGKEYKCKVSNKALPAPIEKTISKAKGQPREPQVYTLPPSREEMTKNQVSLTCLVKGFYPSDIAVEWESNGQPENNYKTTPPVLDSDGSFFLYSKLTVDKSRWQQGNVFSCSVMHEALHNHYTQKSLSLSPGK

SEQ ID NO: 36 - protein, 485 aa, Artificial Sequence
  source: /note="Description of Artificial Sequence: Synthetic polypeptide"
MAETVESCLAKPHTENSFTNVWKEGDSRYANYEGCLWAAGGVVVCTGDEHQCYGTWVPIGLAIPENEGGGSEGGGSEGGGSEGGGTKPPEYGDTPIPGYTYINPLDGTYPPGTEQNPANPNPSLEESQPLNTFMFQGNRFRNRQGALTVYTGTFTQGTDPVKTYYQYTPVSSRAMYDAYWNGKFRDCAFHSGFNEDPFVCEYQGQSSDLPQPPANAGGESGGGSGGGSEGGGSEGGGSEGGGSEGGGSGGGSGSGARSDKTHTCPPCPAPELLGGPSVFLFPPKPKDTLMISRTPEVTCVVVDVSHEDPEVKFNWYVDGVEVHNAKTKPREEQYNSTYRVVSVLTVLHQDWLNGKEYKCKVSNKALPAPIEKTISKAKGQPREPQVYTLPPSREEMTKNQVSLTCLVKGFYPSDIAVEWESNGQPENNYKTTPPVLDSDGSFFLYSKLTVDKSRWQQGNVFSCSVMHEALHNHYTQKSLSLSPGK

SEQ ID NO: 37 - DNA, 765 bp, Artificial Sequence
  source: /note="Description of Artificial Sequence: Synthetic polynucleotide"
atggccgaaaccgtggaatcatgtctggcgaagccccataccgagaactccttcaccaacgtctggaaagagggcgacagccgctacgccaactacgagggctgcctgtggaacgccggtggagtggtcgtctgcaccggggatgagactcagtgctacggacactgggtgcctatcggactggccattcccgagaacgaggggggtggtagcgaaggcggcggatcggaaggcggaggatctgagggagggggaaccaagcctccggaatacggcgacactccgatccccgggtatacgtacatcaatccgctggacgggacctacccgcctggaactgagcagaacccggccaacccaaaccctagcctcgaggaatcccagccgttgaacaccttcatgttccaagggaaccgcttcaggaacagacagggagcgctgaccgtgtacactggcaccttcacacaaggcaccgaccccgtcaagacctactaccagtacactcctgtgtcctcgcgggctatgtacgatgcgtactggaatgggaagtttcgggactgcgctttccactccggcttcaacgaggatccattcgtgtgcgaatatcagggccagagctccgacctcccccaaccccctgcaaacgccggcggagaatccggagggggatcaggaggcggaagcgaagggggtggatccgaaggaggcggatccgagggtggaggctccgaagggggaggctctggtggtggctccggatcggga

SEQ ID NO: 38 - DNA, 765 bp, Artificial Sequence
  source: /note="Description of Artificial Sequence: Synthetic polynucleotide"
atggccgaaaccgtggaatcatgtctggcgaagccccataccgagaactccttcaccaacgtctggaaagagggcgacagccgctacgccaactacgagggctgcctgtggaacgccggtggagtggtcgtctgcaccggggatgagactcagtgctacggacactgggtgcctatcggactggccattcccgagaacgaggggggtggtagcgaaggcggcggatcggaaggcggaggatctgagggagggggaaccaagcctccggaatacggcgacactccgatccccgggtatacgtacatcaatccgctggacgggacctacccgcctggaactgagcagaacccggccaacccaaaccctagcctcgaggaatcccagccgttgaacaccttcatgttccaaaacaaccgcttcaggaacgtgaacggagtgctgaccgtgtacactggcaccttcacacaaggcaccgaccccgtcaagacctactaccagtacactcctgtgtcctcgcgggctatgtacgatgcgtactggaatgggaagtttcgggactgcgctttccactccggcttcaacgaggatccattcgtgtgcgaatatcagggccagagctccgacctcccccaaccccctgcaaacgccggcggagaatccggagggggatcaggaggcggaagcgaagggggtggatccgaaggaggcggatccgagggtggaggctccgaagggggaggctctggtggtggctccggatcggga

SEQ ID NO: 39 - DNA, 765 bp, Artificial Sequence
  source: /note="Description of Artificial Sequence: Synthetic polynucleotide"
atggccgaaaccgtggaatcatgtctggcgaagccccataccgagaactccttcaccaacgtctggaaagagggcgacagccgctacgccaactacgagggctgcctgtggaacgccggtggagtggtcgtctgcaccggggatgagactcagtgctacggacactgggtgcctatcggactggccattcccgagaacgaggggggtggtagcgaaggcggcggatcggaaggcggaggatctgagggagggggaaccaagcctccggaatacggcgacactccgatccccgggtatacgtacatcaatccgctggacgggacctacccgcctggaactgagcagaacccggccaacccaaaccctagcctcgaggaatcccagccgttgaacaccttcatgttccaagggaaccgcttcagggctagacagggagcgctgaccgtgtacactggcaccttcacacaaggcaccgaccccgtcaagacctactaccagtacactcctgtgtcctcgcgggctatgtacgatgcgtactggaatgggaagtttcgggactgcgctttccactccggcttcaacgaggatccattcgtgtgcgaatatcagggccagagctccgacctcccccaaccccctgcaaacgccggcggagaatccggagggggatcaggaggcggaagcgaagggggtggatccgaaggaggcggatccgagggtggaggctccgaagggggaggctctggtggtggctccggatcggga

SEQ ID NO: 40 - DNA, 765 bp, Artificial Sequence
  source: /note="Description of Artificial Sequence: Synthetic polynucleotide"
atggccgaaaccgtggaatcatgtctggcgaagccccataccgagaactccttcaccaacgtctggaaagagggcgacagccgctacgccaactacgagggctgcctgtggaacgccggtggagtggtcgtctgcaccggggatgagactcagtgctacggacactgggtgcctatcggactggccattcccgagaacgaggggggtggtagcgaaggcggcggatcggaaggcggaggatctgagggagggggaaccaagcctccggaatacggcgacactccgatccccgggtatacgtacatcaatccgctggacgggacctacccgcctggaactgagcagaacccggccaacccaaaccctagcctcgaggaatcccagccgttgaacaccttcatgttccaaaacaaccgcttcagggccgtgaacggagtgctgaccgtgtacactggcaccttcacacaaggcaccgaccccgtcaagacctactaccagtacactcctgtgtcctcgcgggctatgtacgatgcgtactggaatgggaagtttcgggactgcgctttccactccggcttcaacgaggatccattcgtgtgcgaatatcagggccagagctccgacctcccccaaccccctgcaaacgccggcggagaatccggagggggatcaggaggcggaagcgaagggggtggatccgaaggaggcggatccgagggtggaggctccgaagggggaggctctggtggtggctccggatcggga

SEQ ID NO: 41 - DNA, 765 bp, Artificial Sequence
  source: /note="Description of Artificial Sequence: Synthetic polynucleotide"
atggccgaaaccgtggaatcatgtctggcgaagccccataccgagaactccttcaccaacgtctggaaagagggcgacagccgctacgccaactacgagggctgcctgtggaacgccggtggagtggtcgtctgcaccggggatgagcaccagtgctacggaacttgggtgcctatcggactggccattcccgagaacgaggggggtggtagcgaaggcggcggatcggaaggcggaggatctgagggagggggaaccaagcctccggaatacggcgacactccgatccccgggtatacgtacatcaatccgctggacgggacctacccgcctggaactgagcagaacccggccaacccaaaccctagcctcgaggaatcccagccgttgaacaccttcatgttccaagggaaccgcttcagggctagacagggagcgctgaccgtgtacactggcaccttcacacaaggcaccgaccccgtcaagacctactaccagtacactcctgtgtcctcgcgggctatgtacgatgcgtactggaatgggaagtttcgggactgcgctttccactccggcttcaacgaggatccattcgtgtgcgaatatcagggccagagctccgacctcccccaaccccctgcaaacgccggcggagaatccggagggggatcaggaggcggaagcgaagggggtggatccgaaggaggcggatccgagggtggaggctccgaagggggaggctctggtggtggctccggatcggga

SEQ ID NO: 42 - DNA, 765 bp, Artificial Sequence
  source: /note="Description of Artificial Sequence: Synthetic polynucleotide"
atggccgaaaccgtggaatcatgtctggcgaagccccataccgagaactccttcaccaacgtctggaaagagggcgacagccgctacgccaactacgagggctgcctgtggaacgccggtggagtggtcgtctgcaccggggatgagcaccagtgctacggaacttgggtgcctatcggactggccattcccgagaacgaggggggtggtagcgaaggcggcggatcggaaggcggaggatctgagggagggggaaccaagcctccggaatacggcgacactccgatccccgggtatacgtacatcaatccgctggacgggacctacccgcctggaactgagcagaacccggccaacccaaaccctagcctcgaggaatcccagccgttgaacaccttcatgttccaaaacaaccgcttcagggccgtgaacggagtgctgaccgtgtacactggcaccttcacacaaggcaccgaccccgtcaagacctactaccagtacactcctgtgtcctcgcgggctatgtacgatgcgtactggaatgggaagtttcgggactgcgctttccactccggcttcaacgaggatccattcgtgtgcgaatatcagggccagagctccgacctcccccaaccccctgcaaacgccggcggagaatccggagggggatcaggaggcggaagcgaagggggtggatccgaaggaggcggatccgagggtggaggctccgaagggggaggctctggtggtggctccggatcggga

SEQ ID NO: 43 - DNA, 765 bp, Artificial Sequence
  source: /note="Description of Artificial Sequence: Synthetic polynucleotide"
atggccgaaaccgtggaatcatgtctggcgaagccccataccgagaactccttcaccaacgtctggaaagagggcgacagccgctacgccaactacgagggctgcctgtggaacgccggtggagtggtcgtctgcaccggggatgagcatcagtgctacggaacctgggtgcctatcggactggccattcccgagaacgaggggggtggtagcgaaggcggcggatcggaaggcggaggatctgagggagggggaaccaagcctccggaatacggcgacactccgatccccgggtatacgtacatcaatccgctggacgggacctacccgcctggaactgagcagaacccggccaacccaaaccctagcctcgaggaatcccagccgttgaacaccttcatgttccaagggaaccgcttcaggaacagacagggagcgctgaccgtgtacactggcaccttcacacaaggcaccgaccccgtcaagacctactaccagtacactcctgtgtcctcgcgggctatgtacgatgcgtactggaatgggaagtttcgggactgcgctttccactccggcttcaacgaggatccattcgtgtgcgaatatcagggccagagctccgacctcccccaaccccctgcaaacgccggcggagaatccggagggggatcaggaggcggaagcgaagggggtggatccgaaggaggcggatccgagggtggaggctccgaagggggaggctctggtggtggctccggatcggga

SEQ ID NO: 44 - DNA, 765 bp, Artificial Sequence
  source: /note="Description of Artificial Sequence: Synthetic polynucleotide"
atggccgaaaccgtggaatcatgtctggcgaagccccataccgagaactccttcaccaacgtctggaaagagggcgacagccgctacgccaactacgagggctgcctgtgggccgccggtggagtggtcgtctgcaccggggatgagcatcagtgctacggaacctgggtgcctatcggactggccattcccgagaacgaggggggtggtagcgaaggcggcggatcggaaggcggaggatctgagggagggggaaccaagcctccggaatacggcgacactccgatccccgggtatacgtacatcaatccgctggacgggacctacccgcctggaactgagcagaacccggccaacccaaaccctagcctcgaggaatcccagccgttgaacaccttcatgttccaagggaaccgcttcaggaacagacagggagcgctgaccgtgtacactggcaccttcacacaaggcaccgaccccgtcaagacctactaccagtacactcctgtgtcctcgcgggctatgtacgatgcgtactggaatgggaagtttcgggactgcgctttccactccggcttcaacgaggatccattcgtgtgcgaatatcagggccagagctccgacctcccccaaccccctgcaaacgccggcggagaatccggagggggatcaggaggcggaagcgaagggggtggatccgaaggaggcggatccgagggtggaggctccgaagggggaggctctggtggtggctccggatcggga

SEQ ID NO: 45 - DNA, 1458 bp, Artificial Sequence
  source: /note="Description of Artificial Sequence: Synthetic polynucleotide"
atggccgaaaccgtggaatcatgtctggcgaagccccataccgagaactccttcaccaacgtctggaaagagggcgacagccgctacgccaactacgagggctgcctgtggaacgccggtggagtggtcgtctgcaccggggatgagactcagtgctacggacactgggtgcctatcggactggccattcccgagaacgaggggggtggtagcgaaggcggcggatcggaaggcggaggatctgagggagggggaaccaagcctccggaatacggcgacactccgatccccgggtatacgtacatcaatccgctggacgggacctacccgcctggaactgagcagaacccggccaacccaaaccctagcctcgaggaatcccagccgttgaacaccttcatgttccaagggaaccgcttcaggaacagacagggagcgctgaccgtgtacactggcaccttcacacaaggcaccgaccccgtcaagacctactaccagtacactcctgtgtcctcgcgggctatgtacgatgcgtactggaatgggaagtttcgggactgcgctttccactccggcttcaacgaggatccattcgtgtgcgaatatcagggccagagctccgacctcccccaaccccctgcaaacgccggcggagaatccggagggggatcaggaggcggaagcgaagggggtggatccgaaggaggcggatccgagggtggaggctccgaagggggaggctctggtggtggctccggatcgggagccagatctgacaaaactcacacatgcccaccgtgcccagcacctgaactcctggggggaccgtcagtcttcctcttccccccaaaacccaaggacaccctcatgatctcccggacccctgaggtcacatgcgtggtggtggacgtgagccacgaagaccctgaggtcaagttcaactggtacgtggacggcgtggaggtgcataatgccaagacaaagccgcgggaggagcagtacaacagcacgtaccgtgtggtcagcgtcctcaccgtcctgcaccaggactggctgaatggcaaggagtacaagtgcaaggtctccaacaaagccctcccagcccccatcgagaaaaccatctccaaagccaaagggcagccccgagaaccacaggtgtacaccctgcccccatcccgggaggagatgaccaagaaccaggtcagcctgacctgcctggtcaaaggcttctatcccagcgacatcgccgtggagtgggagagcaatgggcagccggagaacaactacaagaccacgcctcccgtgctggactccgacggctccttcttcctctacagcaagctcaccgtggacaagagcaggtggcagcaggggaacgtcttctcatgctccgtgatgcacgaggctctgcacaaccactacacgcagaagagcctctccctgtctccgggtaaatga

SEQ ID NO: 46 - DNA, 1458 bp, Artificial Sequence
  source: /note="Description of Artificial Sequence: Synthetic polynucleotide"
atggccgaaaccgtggaatcatgtctggcgaagccccataccgagaactccttcaccaacgtctggaaagagggcgacagccgctacgccaactacgagggctgcctgtggaacgccggtggagtggtcgtctgcaccggggatgagactcagtgctacggacactgggtgcctatcggactggccattcccgagaacgaggggggtggtagcgaaggcggcggatcggaaggcggaggatctgagggagggggaaccaagcctccggaatacggcgacactccgatccccgggtatacgtacatcaatccgctggacgggacctacccgcctggaactgagcagaacccggccaacccaaaccctagcctcgaggaatcccagccgttgaacaccttcatgttccaaaacaaccgcttcaggaacgtgaacggagtgctgaccgtgtacactggcaccttcacacaaggcaccgaccccgtcaagacctactaccagtacactcctgtgtcctcgcgggctatgtacgatgcgtactggaatgggaagtttcgggactgcgctttccactccggcttcaacgaggatccattcgtgtgcgaatatcagggccagagctccgacctcccccaaccccctgcaaacgccggcggagaatccggagggggatcaggaggcggaagcgaagggggtggatccgaaggaggcggatccgagggtggaggctccgaagggggaggctctggtggtggctccggatcgggagccagatctgacaaaactcacacatgcccaccgtgcccagcacctgaactcctggggggaccgtcagtcttcctcttccccccaaaacccaaggacaccctcatgatctcccggacccctgaggtcacatgcgtggtggtggacgtgagccacgaagaccctgaggtcaagttcaactggtacgtggacggcgtggaggtgcataatgccaagacaaagccgcgggaggagcagtacaacagcacgtaccgtgtggtcagcgtcctcaccgtcctgcaccaggactggctgaatggcaaggagtacaagtgcaaggtctccaacaaagccctcccagcccccatcgagaaaaccatctccaaagccaaagggcagccccgagaaccacaggtgtacaccctgcccccatcccgggaggagatgaccaagaaccaggtcagcctgacctgcctggtcaaaggcttctatcccagcgacatcgccgtggagtgggagagcaatgggcagccggagaacaactacaagaccacgcctcccgtgctggactccgacggctccttcttcctctacagcaagctcaccgtggacaagagcaggtggcagcaggggaacgtcttctcatgctccgtgatgcacgaggctctgcacaaccactacacgcagaagagcctctccctgtctccgggtaaatga

SEQ ID NO: 47 - DNA, 1458 bp, Artificial Sequence
  source: /note="Description of Artificial Sequence: Synthetic polynucleotide"
atggccgaaaccgtggaatcatgtctggcgaagccccataccgagaactccttcaccaacgtctggaaagagggcgacagccgctacgccaactacgagggctgcctgtggaacgccggtggagtggtcgtctgcaccggggatgagactcagtgctacggacactgggtgcctatcggactggccattcccgagaacgaggggggtggtagcgaaggcggcggatcggaaggcggaggatctgagggagggggaaccaagcctccggaatacggcgacactccgatccccgggtatacgtacatcaatccgctggacgggacctacccgcctggaactgagcagaacccggccaacccaaaccctagcctcgaggaatcccagccgttgaacaccttcatgttccaagggaaccgcttcagggctagacagggagcgctgaccgtgtacactggcaccttcacacaaggcaccgaccccgtcaagacctactaccagtacactcctgtgtcctcgcgggctatgtacgatgcgtactggaatgggaagtttcgggactgcgctttccactccggcttcaacgaggatccattcgtgtgcgaatatcagggccagagctccgacctcccccaaccccctgcaaacgccggcggagaatccggagggggatcaggaggcggaagcgaagggggtggatccgaaggaggcggatccgagggtggaggctccgaagggggaggctctggtggtggctccggatcgggagccagatctgacaaaactcacacatgcccaccgtgcccagcacctgaactcctggggggaccgtcagtcttcctcttccccccaaaacccaaggacaccctcatgatctcccggacccctgaggtcacatgcgtggtggtggacgtgagccacgaagaccctgaggtcaagttcaactggtacgtggacggcgtggaggtgcataatgccaagacaaagccgcgggaggagcagtacaacagcacgtaccgtgtggtcagcgtcctcaccgtcctgcaccaggactggctgaatggcaaggagtacaagtgcaaggtctccaacaaagccctcccagcccccatcgagaaaaccatctccaaagccaaagggcagccccgagaaccacaggtgtacaccctgcccccatcccgggaggagatgaccaagaaccaggtcagcctgacctgcctggtcaaaggcttctatcccagcgacatcgccgtggagtgggagagcaatgggcagccggagaacaactacaagaccacgcctcccgtgctggactccgacggctccttcttcctctacagcaagctcaccgtggacaagagcaggtggcagcaggggaacgtcttctcatgctccgtgatgcacgaggctctgcacaaccactacacgcagaagagcctctccctgtctccgggtaaatga

SEQ ID NO: 48 - DNA, 1458 bp, Artificial Sequence
  source: /note="Description of Artificial Sequence: Synthetic polynucleotide"
atggccgaaaccgtggaatcatgtctggcgaagccccataccgagaactccttcaccaacgtctggaaagagggcgacagccgctacgccaactacgagggctgcctgtggaacgccggtggagtggtcgtctgcaccggggatgagactcagtgctacggacactgggtgcctatcggactggccattcccgagaacgaggggggtggtagcgaaggcggcggatcggaaggcggaggatctgagggagggggaaccaagcctccggaatacggcgacactccgatccccgggtatacgtacatcaatccgctggacgggacctacccgcctggaactgagcagaacccggccaacccaaaccctagcctcgaggaatcccagccgttgaacaccttcatgttccaaaacaaccgcttcagggccgtgaacggagtgctgaccgtgtacactggcaccttcacacaaggcaccgaccccgtcaagacctactaccagtacactcctgtgtcctcgcgggctatgtacgatgcgtactggaatgggaagtttcgggactgcgctttccactccggcttcaacgaggatccattcgtgtgcgaatatcagggccagagctccgacctcccccaaccccctgcaaacgccggcggagaatccggagggggatcaggaggcggaagcgaagggggtggatccgaaggaggcggatccgagggtggaggctccgaagggggaggctctggtggtggctccggatcgggagccagatctgacaaaactcacacatgcccaccgtgcccagcacctgaactcctggggggaccgtcagtcttcctcttccccccaaaacccaaggacaccctcatgatctcccggacccctgaggtcacatgcgtggtggtggacgtgagccacgaagaccctgaggtcaagttcaactggtacgtggacggcgtggaggtgcataatgccaagacaaagccgcgggaggagcagtacaacagcacgtaccgtgtggtcagcgtcctcaccgtcctgcaccaggactggctgaatggcaaggagtacaagtgcaaggtctccaacaaagccctcccagcccccatcgagaaaaccatctccaaagccaaagggcagccccgagaaccacaggtgtacaccctgcccccatcccgggaggagatgaccaagaaccaggtcagcctgacctgcctggtcaaaggcttctatcccagcgacatcgccgtggagtgggagagcaatgggcagccggagaacaactacaagaccacgcctcccgtgctggactccgacggctccttcttcctctacagcaagctcaccgtggacaagagcaggtggcagcaggggaacgtcttctcatgctccgtgatgcacgaggctctgcacaaccactacacgcagaagagcctctccctgtctccgggtaaatga

SEQ ID NO: 49 - DNA, 1458 bp, Artificial Sequence
  source: /note="Description of Artificial Sequence: Synthetic polynucleotide"
atggccgaaaccgtggaatcatgtctggcgaagccccataccgagaactccttcaccaacgtctggaaagagggcgacagccgctacgccaactacgagggctgcctgtggaacgccggtggagtggtcgtctgcaccggggatgagcaccagtgctacggaacttgggtgcctatcggactggccattcccgagaacgaggggggtggtagcgaaggcggcggatcggaaggcggaggatctgagggagggggaaccaagcctccggaatacggcgacactccgatccccgggtatacgtacatcaatccgctggacgggacctacccgcctggaactgagcagaacccggccaacccaaaccctagcctcgaggaatcccagccgttgaacaccttcatgttccaagggaaccgcttcagggctagacagggagcgctgaccgtgtacactggcaccttcacacaaggcaccgaccccgtcaagacctactaccagtacactcctgtgtcctcgcgggctatgtacgatgcgtactggaatgggaagtttcgggactgcgctttccactccggcttcaacgaggatccattcgtgtgcgaatatcagggccagagctccgacctcccccaaccccctgcaaacgccggcggagaatccggagggggatcaggaggcggaagcgaagggggtggatccgaaggaggcggatccgagggtggaggctccgaagggggaggctctggtggtggctccggatcgggagccagatctgacaaaactcacacatgcccaccgtgcccagcacctgaactcctggggggaccgtcagtcttcctcttccccccaaaacccaaggacaccctcatgatctcccggacccctgaggtcacatgcgtggtggtggacgtgagccacgaagaccctgaggtcaagttcaactggtacgtggacggcgtggaggtgcataatgccaagacaaagccgcgggaggagcagtacaacagcacgtaccgtgtggtcagcgtcctcaccgtcctgcaccaggactggctgaatggcaaggagtacaagtgcaaggtctccaacaaagccctcccagcccccatcgagaaaaccatctccaaagccaaagggcagccccgagaaccacaggtgtacaccctgcccccatcccgggaggagatgaccaagaaccaggtcagcctgacctgcctggtcaaaggcttctatcccagcgacatcgccgtggagtgggagagcaatgggcagccggagaacaactacaagaccacgcctcccgtgctggactccgacggctccttcttcctctacagcaagctcaccgtggacaagagcaggtggcagcaggggaacgtcttctcatgctccgtgatgcacgaggctctgcacaaccactacacgcagaagagcctctccctgtctccgggtaaatga

SEQ ID NO: 50 - DNA, 1458 bp, Artificial Sequence
  source: /note="Description of Artificial Sequence: Synthetic polynucleotide"
atggccgaaaccgtggaatcatgtctggcgaagccccataccgagaactccttcaccaacgtctggaaagagggcgacagccgctacgccaactacgagggctgcctgtggaacgccggtggagtggtcgtctgcaccggggatgagcaccagtgctacggaacttgggtgcctatcggactggccattcccgagaacgaggggggtggtagcgaaggcggcggatcggaaggcggaggatctgagggagggggaaccaagcctccggaatacggcgacactccgatccccgggtatacgtacatcaatccgctggacgggacctacccgcctggaactgagcagaacccggccaacccaaaccctagcctcgaggaatcccagccgttgaacaccttcatgttccaaaacaaccgcttcagggccgtgaacggagtgctgaccgtgtacactggcaccttcacacaaggcaccgaccccgtcaagacctactaccagtacactcctgtgtcctcgcgggctatgtacgatgcgtactggaatgggaagtttcgggactgcgctttccactccggcttcaacgaggatccattcgtgtgcgaatatcagggccagagctccgacctcccccaaccccctgcaaacgccggcggagaatccggagggggatcaggaggcggaagcgaagggggtggatccgaaggaggcggatccgagggtggaggctccgaagggggaggctctggtggtggctccggatcgggagccagatctgacaaaactcacacatgcccaccgtgcccagcacctgaactcctggggggaccgtcagtcttcctcttccccccaaaacccaaggacaccctcatgatctcccggacccctgaggtcacatgcgtggtggtggacgtgagccacgaagaccctgaggtcaagttcaactggtacgtggacggcgtggaggtgcataatgccaagacaaagccgcgggaggagcagtacaacagcacgtaccgtgtggtcagcgtcctcaccgtcctgcaccaggactggctgaatggcaaggagtacaagtgcaaggtctccaacaaagccctcccagcccccatcgagaaaaccatctccaaagccaaagggcagccccgagaaccacaggtgtacaccctgcccccatcccgggaggagatgaccaagaaccaggtcagcctgacctgcctggtcaaaggcttctatcccagcgacatcgccgtggagtgggagagcaatgggcagccggagaacaactacaagaccacgcctcccgtgctggactccgacggctccttcttcctctacagcaagctcaccgtggacaagagcaggtggcagcaggggaacgtcttctcatgctccgtgatgcacgaggctctgcacaaccactacacgcagaagagcctctccctgtctccgggtaaatga

SEQ ID NO: 51 - DNA, 1458 bp, Artificial Sequence
  source: /note="Description of Artificial Sequence: Synthetic polynucleotide"
atggccgaaaccgtggaatcatgtctggcgaagccccataccgagaactccttcaccaacgtctggaaagagggcgacagccgctacgccaactacgagggctgcctgtggaacgccggtggagtggtcgtctgcactggggatgagcaccagtgctacggaacctgggtgcctatcggactggccattcccgagaacgaggggggtggtagcgaaggcggcggatcggaaggcggaggatctgagggagggggaaccaagcctccggaatacggcgacactccgatccccgggtatacgtacatcaatccgctggacgggacctacccgcctggaactgagcagaacccggccaacccaaaccctagcctcgaggaatcccagccgttgaacaccttcatgttccaagggaaccgcttcaggaacagacagggagcgctgaccgtgtacactggcaccttcacacaaggcaccgaccccgtcaagacctactaccagtacactcctgtgtcctcgcgggctatgtacgatgcgtactggaatgggaagtttcgggactgcgctttccactccggcttcaacgaggatccattcgtgtgcgaatatcagggccagagctccgacctcccccaaccccctgcaaacgccggcggagaatccggagggggatcaggaggcggaagcgaagggggtggatccgaaggaggcggatccgagggtggaggctccgaagggggaggctctggtggtggctccggatcgggagccagatctgacaaaactcacacatgcccaccgtgcccagcacctgaactcctggggggaccgtcagtcttcctcttccccccaaaacccaaggacaccctcatgatctcccggacccctgaggtcacatgcgtggtggtggacgtgagccacgaagaccctgaggtcaagttcaactggtacgtggacggcgtggaggtgcataatgccaagacaaagccgcgggaggagcagtacaacagcacgtaccgtgtggtcagcgtcctcaccgtcctgcaccaggactggctgaatggcaaggagtacaagtgcaaggtctccaacaaagccctcccagcccccatcgagaaaaccatctccaaagccaaagggcagccccgagaaccacaggtgtacaccctgcccccatcccgggaggagatgaccaagaaccaggtcagcctgacctgcctggtcaaaggcttctatcccagcgacatcgccgtggagtgggagagcaatgggcagccggagaacaactacaagaccacgcctcccgtgctggactccgacggctccttcttcctctacagcaagctcaccgtggacaagagcaggtggcagcaggggaacgtcttctcatgctccgtgatgcacgaggctctgcacaaccactacacgcagaagagcctctccctgtctccgggtaaatga

SEQ ID NO: 52 - DNA, 1458 bp, Artificial Sequence
  source: /note="Description of Artificial Sequence: Synthetic polynucleotide"
atggccgaaaccgtggaatcatgtctggcgaagccccataccgagaactccttcaccaacgtctggaaagagggcgacagccgctacgccaactacgagggctgcctgtgggccgccggtggagtggtcgtctgcactggggatgagcaccagtgctacggaacctgggtgcctatcggactggccattcccgagaacgaggggggtggtagcgaaggcggcggatcggaaggcggaggatctgagggagggggaaccaagcctccggaatacggcgacactccgatccccgggtatacgtacatcaatccgctggacgggacctacccgcctggaactgagcagaacccggccaacccaaaccctagcctcgaggaatcccagccgttgaacaccttcatgttccaagggaaccgcttcaggaacagacagggagcgctgaccgtgtacactggcaccttcacacaaggcaccgaccccgtcaagacctactaccagtacactcctgtgtcctcgcgggctatgtacgatgcgtactggaatgggaagtttcgggactgcgctttccactccggcttcaacgaggatccattcgtgtgcgaatatcagggccagagctccgacctcccccaaccccctgcaaacgccggcggagaatccggagggggatcaggaggcggaagcgaagggggtggatccgaaggaggcggatccgagggtggaggctccgaagggggaggctctggtggtggctccggatcgggagccagatctgacaaaactcacacatgcccaccgtgcccagcacctgaactcctggggggaccgtcagtcttcctcttccccccaaaacccaaggacaccctcatgatctcccggacccctgaggtcacatgcgtggtggtggacgtgagccacgaagaccctgaggtcaagttcaactggtacgtggacggcgtggaggtgcataatgccaagacaaagccgcgggaggagcagtacaacagcacgtaccgtgtggtcagcgtcctcaccgtcctgcaccaggactggctgaatggcaaggagtacaagtgcaaggtctccaacaaagccctcccagcccccatcgagaaaaccatctccaaagccaaagggcagccccgagaaccacaggtgtacaccctgcccccatcccgggaggagatgaccaagaaccaggtcagcctgacctgcctggtcaaaggcttctatcccagcgacatcgccgtggagtgggagagcaatgggcagccggagaacaactacaagaccacgcctcccgtgctggactccgacggctccttcttcctctacagcaagctcaccgtggacaagagcaggtggcagcaggggaacgtcttctcatgctccgtgatgcacgaggctctgcacaaccactacacgcagaagagcctctccctgtctccgggtaaatga

SEQ ID NO: 53 - protein, 6 aa, Artificial Sequence
  source: /note="Description of Artificial Sequence: Synthetic 6xHis tag"
HHHHHH

SEQ ID NO: 54 - protein, 4 aa, Artificial Sequence
  source: /note="Description of Artificial Sequence: Synthetic peptide"
EDGS